European Patent Specification EP 3 701 966 B1, published July 9, 2025. Title: MEDICAMENTS AND METHODS FOR TREATING HEPATITIS B VIRUS-RELATED LIVER DISEASES USING SUFFICIENT DOSAGE. Applicant: SHANGHAI HEP PHARMACEUTICAL CO., LTD. The sequence listing filed with the application follows.

SEQUENCE LISTING (51 sequences)

SEQ ID NO: 1 - protein, 60 aa, Artificial Sequence
  PEPTIDE (1)..(60): Description of Artificial Sequence: Synthetic polypeptide
  MYRISTATE (1)..(1): N-term Myr
  AMIDATION (60)..(60): C-term NH2
GTNLSVPNPLGFFPDHQLDPAFGANSNNPDWDFNPNKDHWPEANQVGAGAFGPGFTPPHG

SEQ ID NO: 2 - protein, 55 aa, Artificial Sequence
  PEPTIDE (1)..(55): Description of Artificial Sequence: Synthetic polypeptide
  MYRISTATE (1)..(1): N-term Myr
  AMIDATION (55)..(55): C-term NH2
GTNLSVPNPLGFFPDHQLDPAFGANSNNPDWDFNPNKDHWPEANQVGAGAFGPGF

SEQ ID NO: 3 - protein, 47 aa, Artificial Sequence
  PEPTIDE (1)..(47): Description of Artificial Sequence: Synthetic polypeptide
  MYRISTATE (1)..(1): N-term Myr
  AMIDATION (47)..(47): C-term NH2
GTNLSVPNPLGFFPDHQLDPAFGANSNNPDWDFNPNKDHWPEANQVG

SEQ ID NO: 4 - protein, 40 aa, Artificial Sequence
  PEPTIDE (1)..(40): Description of Artificial Sequence: Synthetic polypeptide
  MYRISTATE (1)..(1): N-term Myr
  AMIDATION (40)..(40): C-term NH2
GTNLSVPNPLGFFPDHQLDPAFGANSNNPDWDFNPNKDHW

SEQ ID NO: 5 - protein, 35 aa, Artificial Sequence
  PEPTIDE (1)..(35): Description of Artificial Sequence: Synthetic polypeptide
  MYRISTATE (1)..(1): N-term Myr
  AMIDATION (35)..(35): C-term NH2
GTNLSVPNPLGFFPDHQLDPAFGANSNNPDWDFNP

SEQ ID NO: 6 - protein, 30 aa, Artificial Sequence
  PEPTIDE (1)..(30): Description of Artificial Sequence: Synthetic polypeptide
  MYRISTATE (1)..(1): N-term Myr
  ACETYLATION (30)..(30): C-term NH2
GTNLSVPNPLGFFPDHQLDPAFGANSNNPD

SEQ ID NO: 7 - protein, 25 aa, Artificial Sequence
  PEPTIDE (1)..(25): Description of Artificial Sequence: Synthetic peptide
  MYRISTATE (1)..(1): N-term Myr
  AMIDATION (25)..(25): C-term NH2
GTNLSVPNPLGFFPDHQLDPAFGAN

SEQ ID NO: 8 - protein, 20 aa, Artificial Sequence
  PEPTIDE (1)..(20): Description of Artificial Sequence: Synthetic peptide
  MYRISTATE (1)..(1): N-term Myr
  AMIDATION (20)..(20): C-term NH2
GTNLSVPNPLGFFPDHQLDP

SEQ ID NO: 9 - protein, 58 aa, Artificial Sequence
  PEPTIDE (1)..(58): Description of Artificial Sequence: Synthetic polypeptide
  MYRISTATE (1)..(1): N-term Myr
  AMIDATION (58)..(58): C-term NH2
GGWSSKPRQGMGTNLSVPNPLGFFPDHQLDPAFGANSNNPDWDFNPNKDHWPEANQVG

SEQ ID NO: 10 - protein, 57 aa, Artificial Sequence
  PEPTIDE (1)..(57): Description of Artificial Sequence: Synthetic polypeptide
  MYRISTATE (1)..(1): N-term Myr
  AMIDATION (57)..(57): C-term NH2
GLSWTVPLEWGTNLSVPNPLGFFPDHQLDPAFGANSNNPDWDFNPNKDHWPEANQVG

SEQ ID NO: 11 - protein, 47 aa, Artificial Sequence; identical to SEQ ID NO: 3
  PEPTIDE (1)..(47): Description of Artificial Sequence: Synthetic polypeptide
  PALMITATE (1)..(1): N-term Plam
  AMIDATION (47)..(47): C-term NH2

SEQ ID NO: 12 - protein, 47 aa, Artificial Sequence; identical to SEQ ID NO: 3
  PEPTIDE (1)..(47): Description of Artificial Sequence: Synthetic polypeptide
  ACETYLATION (1)..(1): N-term Stearoyl
  AMIDATION (47)..(47): C-term NH2

SEQ ID NO: 13 - protein, 47 aa, Artificial Sequence; identical to SEQ ID NO: 3
  PEPTIDE (1)..(47): Description of Artificial Sequence: Synthetic polypeptide
  ACETYLATION (1)..(1): N-term Chol
  AMIDATION (47)..(47): C-term NH2

SEQ ID NO: 14 - protein, 47 aa, Artificial Sequence
  PEPTIDE (1)..(47): Description of Artificial Sequence: Synthetic polypeptide
  MYRISTATE (1)..(1): N-term Myr
  AMIDATION (47)..(47): C-term NH2
GTNLSVPNPLGFFPDHQLDPAFGANSNNPDWDFNPVKDDWPAANQVG

SEQ ID NO: 15 - protein, 47 aa, Artificial Sequence
  PEPTIDE (1)..(47): Description of Artificial Sequence: Synthetic polypeptide
  MYRISTATE (1)..(1): N-term Myr
  AMIDATION (47)..(47): C-term NH2
GTNLSVPNPLGFFPDHQLDPAFKANSENPDWDLNPNKDNWPDANKVG

SEQ ID NO: 16 - protein, 47 aa, Artificial Sequence
  MYRISTATE (1)..(1): N-term Myr
  AMIDATION (47)..(47): C-term NH2
  PEPTIDE (1)..(47): Description of Artificial Sequence: Synthetic polypeptide
GQNLSTSNPLGFFPDHQLDPAFRANTANPDWDFNPNKDTWPDANKVG

SEQ ID NO: 17 - protein, 47 aa, Artificial Sequence
  PEPTIDE (1)..(47): Description of Artificial Sequence: Synthetic polypeptide
  MYRISTATE (1)..(1): N-term Myr
  AMIDATION (47)..(47): C-term NH2
GKNISTTNPLGFFPDHQLDPAFRANTRNPDWDHNPNKDHWTEANKVG

SEQ ID NO: 18 - protein, 47 aa, Artificial Sequence
  PEPTIDE (1)..(47): Description of Artificial Sequence: Synthetic polypeptide
  MYRISTATE (1)..(1): N-term Myr
  AMIDATION (47)..(47): C-term NH2
GQNLSVPNPLGFFPDHQLDPLFRANSSSPDWDFNTNKDSWPMANKVG

SEQ ID NO: 19 - protein, 47 aa, Artificial Sequence
  PEPTIDE (1)..(47): Description of Artificial Sequence: Synthetic polypeptide
  MYRISTATE (1)..(1): N-term Myr
  AMIDATION (47)..(47): C-term NH2
GKNLSASNPLGFLPDHQLDPAFRANTNNPDWDFNPKKDPWPEANKVG

SEQ ID NO: 20 - protein, 47 aa, Artificial Sequence
  PEPTIDE (1)..(47): Description of Artificial Sequence: Synthetic polypeptide
  MYRISTATE (1)..(1): N-term Myr
  AMIDATION (47)..(47): C-term NH2
GQNLSVPNPLGFFPDHQLDPLFRANSSSPDWDFNTNKDNWPMANKVG

SEQ ID NO: 21 - protein, 60 aa, Hepatitis B virus; identical to SEQ ID NO: 1

SEQ ID NO: 22 - protein, 55 aa, Hepatitis B virus; identical to SEQ ID NO: 2

SEQ ID NO: 23 - protein, 47 aa, Hepatitis B virus; identical to SEQ ID NO: 3

SEQ ID NO: 24 - protein, 40 aa, Hepatitis B virus; identical to SEQ ID NO: 4

SEQ ID NO: 25 - protein, 35 aa, Hepatitis B virus; identical to SEQ ID NO: 5

SEQ ID NO: 26 - protein, 30 aa, Hepatitis B virus; identical to SEQ ID NO: 6

SEQ ID NO: 27 - protein, 25 aa, Hepatitis B virus
GTNLSVPNPLGFFPDHQLDPAFGAN

SEQ ID NO: 28 - protein, 20 aa, Hepatitis B virus
GTNLSVPNPLGFFPDHQLDP

SEQ ID NO: 29 - protein, 58 aa, Hepatitis B virus; identical to SEQ ID NO: 9

SEQ ID NO: 30 - protein, 57 aa, Hepatitis B virus; identical to SEQ ID NO: 10

SEQ ID NO: 31 - protein, 47 aa, Hepatitis B virus; identical to SEQ ID NO: 3

SEQ ID NO: 32 - protein, 47 aa, Hepatitis B virus; identical to SEQ ID NO: 3

SEQ ID NO: 33 - protein, 47 aa, Hepatitis B virus; identical to SEQ ID NO: 3

SEQ ID NO: 34 - protein, 47 aa, Hepatitis B virus; identical to SEQ ID NO: 14

SEQ ID NO: 35 - protein, 47 aa, Hepatitis B virus; identical to SEQ ID NO: 15

SEQ ID NO: 36 - protein, 47 aa, Hepatitis B virus; identical to SEQ ID NO: 16

SEQ ID NO: 37 - protein, 47 aa, Hepatitis B virus; identical to SEQ ID NO: 17

SEQ ID NO: 38 - protein, 47 aa, Hepatitis B virus; identical to SEQ ID NO: 18

SEQ ID NO: 39 - protein, 47 aa, Hepatitis B virus; identical to SEQ ID NO: 19

SEQ ID NO: 40 - protein, 47 aa, Hepatitis B virus; identical to SEQ ID NO: 20

SEQ ID NO: 41 - DNA, 3221 bp, Hepatitis B virus
ttccactgccttccaccaagctctgcaggatcccaaagtcaggggtctgtattttcctgctggtggctccagttcaggaacagtcaaccctgctccaaatattgcctctcacatctcgtcaatctccgcgaggactggggaccctgtgccgaacatggagaacatcacatcaggattcctaggacccctgctcgtgttacaggcggggtttttcttgttgacaagaatcctcacaataccgcagagtctagactcgtggtggacttctctcaattttctagggggatcacccgtgtgtcttggccaaaattcgcagtccccaacctccaatcactcaccaacctcctgtcctccaatttgtcctggttatcgctggatgtgtctgcggcgttttatcatattcctcttcatcctgctgctatgcctcatcttcttattggttcttctggattatcaaggtatgttgcccgtttgtcctctaattccaggatcaacaacaaccagtacgggaccatgcaaaacctgcacgactcctgctcaaggcaactctatgtttccctcatgttgctgtacaaaacctatggatggaaattgcacctgtattcccatcccatcgtcctgggctttcgcaaaatacctatgggagtgggcctcagtccgtttctcttggctcagtttactagtgccatttgttcagtggttcgtagggctttcccccactgtttggctttcagctatatggatgatgtggtattgggggccaagtctgtacagcatcgtgagtccctttataccgctgttaccaattttcttttgtctctgggtatacatttaaaccctaacaaaacaaaaagatggggttattccctaaacttcatggtctacataattggaagttggggaacgttgccacaggatcatattgtacaaaagatcaaacactgttttagaaaacttcctgttaacagacctattgattggaaagtatgtcaaagaattgtgggtcttttgggctttgctgctccatttactcaatgtggatatcctgccttaatgcctttgtatgcatgtatacaagctaaacaggcttttactttctcgccaacttacaaggcctttctaagtaaacagtatatgaacctttaccccgttgctcggcaacggcctggtctgtgccaagtgtttgctgacgcaacccccactggctggggcttggccataggccatcagcgcatgcgtggaacctttgtggctcctctgccgatccatactgcggaactcctagccgcttgttttgctcgcagccggtctggagcaaagctcatcggaactgataattctgtcgtcctctcgcggaaatatacatcgtttccatggctgctaggctgtactgccaactggatccttcgcgggacgtcctttgtttacgtcccgtcggcgctgaatcccgcggacgacccctcgcggggccgcttgggagtctctcgtccccttctccgtctgccgttccagccgaccacggggcgcacctctctttacgcggtctccccgtctgtgccttctcatctgccggtccgtgtgcacttcgcttcacctctgcacgttgcatggagaccaccgtgaacgcccatcagatcctgcccaaggtcttacataagaggactcttggactctcagcaatgtcaatgaccgaccttgaggcctacttcaaagactgtgtgtttaaggactgggaggagcttggggaggagattaggttaaaggtgtttgtattaggaggctgtaggcataaattggtctgcgcaccagcaccatgcaactttttcacctctgcctaatcatctcttgtacatgtcccacttttcaagcctccaagctgtgccttgggtggctttggggcatggacattgacccttataaagaatttggagctactgtggagttactctcgtttttgccttctgacttctttccttccgtcagagatctcctagacaccgcctcagctctgtatcgagaagccttagagtctcctgagcattgctctcctcaccatactgcactcaggcaagccattctctgctgggtggaattgatgactctagccacctgggtgggtaataatttggaagatccagcatccagggatctagtagtcaattatgttaatactaacatgggtttaaagatcaggcaactattgtggtttcatatatcttgtcttacttttggaagacagactgtgctagaatatttggtctctttcggagtgtggattcgcactcctccagcttatagaccaccaaatgcccctatcttatcaacacttccggagactactgttgttagacgacgggaccgaggcaggtcccctagaagaagaactccctcgcctcgcagacgcagatctcaatcgccgcgtcgcagaagatctcaatctcgggaatctcaatgttagtattccttggactcataaggtgggaaattttactgggctttattcctctacagtacctatctttaatcctgaatggcaaactccttcctttcctaagattcatttacaagaggacattattaataggtgtcaacaatttgtgggccctctcactgtaaatgaaaagagaagactgaaattaattatgcctgccagattctatcctacccacactaaatatttgcccttagacaaaggaattaaaccttattatccagatcaggtagttaatcattacttccaaaccagacattatttacatactctttggaaggctgggattctatataagagggaaaccacacgtagcgcatcattttgcgggtcaccatattcttgggaacaagagctacatcatgggaggttggtcatcaaaacctcgcaaaggcatggggacgaacctttctgttcccaaccctctgggattctttcccgatcatcagttggaccctgcattcggagccaattcaaacaatccagattgggacttcaaccccatcaaggaccactggccagcaggcaaccaggtaggagtgggagcattcgggccaaggctcacccctccacacggcggtattttggggtggagccctcaggctcagggcatattggccacagtgtcaacaattcctcctcctgcctccaccaatcggcagtcaggaaggcagcctactcccatctctccacctctaagagacagtcatcctgaggccatgcagtggaa

SEQ ID NO: 42 - DNA, 3215 bp, Hepatitis B virus
aactccaccactttccaccaaactcttcaagatcccagagtcagggccctgtaccttcctgctggtggctccagttcagaaatagtgagccctgctcagaatactgtctctgccatatcgtcaatcttatcgaagactggggaccctgtaccgaacatggagaacatcgcatcaggactcctaggacccctgctcgtgttacaggcggggtttttcttgttgacaaaaatcctcacaataccacagagtctagactcgtggtggacttctctcaattttctagggggaacacccgtgtgtcttggccaaaattcgcagtcccaaatctccagtcactcaccaacctgttgtcctccaatttgtcctgggtatcgctggatgtgtctgcggcgttttatcatattcctctgcatcctgctgctatgcctcatcttcttgttggttcttctggactatcaaggtatgttgcccgtttgtcctctaattccaggatcatcaacaaccagcaccggaccatgcaaaacctgcacaactcctgctcaaggaacctctatgtttccctcatgttgctgtacaaaacctacggacggaaactgcacctgtattcccatcccatcatcttgggctttcgcaaaattcctatgggagtgggcctcagtccgtttctcttggctcagtttactagtgccatttgttcagtggttcgtagggctttcccccactgtctggctttcagttatatcgatgatgtggttttgggggccaagtctgtacaacatcttgagtccctttataccgctgttaccaattttcttttgtctttgggtatacatttaaaccctcacaaaacaaaaagatggggatattcccttaacttcatgggatatgtaattgggagttggggcacattgccacaggaacatattgtacaaaaaatcaaaatgtgttttaagaaacttcctgtaaacaggcctattgattggaaagtatgtcaacgaattgtgggtcttttggggtttgccgccccttttacgcaatgtggatatcctgctttaatgcctttatatgcatgtatacaagcaaaacaggcttttactttctcgccaacttacaaggcctttctaagtaaacagtatatgaacctttaccccgttgctcggcaacggcctggtctgtgccaagtgtttgctgacgcaacccccactggttggggcttggccattggccatcagcgcatgcgtgggacctttgtgtctcctctgccgatccatactgcggaactcctagccgcttgttttgctcgcagcaggtctggggcaaaactcatcgggactgacaattctgtcgtgctctcccgcaagtatacatcatttccatggctgctaggctgtgctgccaactggatcctgcgcgggacgtcctttgtttacgtcccgtcggcgctgaatcccgcggacgacccctcccggggccgcttggggctctaccgcccgcttctccgcctgttgtaccgaccgaccacggggcgcacctctctttacgcggactccccgtctgtgccttctcatctgccggaccgtgtgcacttcgcttcacctctgcacgtcgcatggagaccaccgtgaacgcccacaggaacctgcccaaggtcttgcataagaggactcttggactttcagcaatgtcaacgaccgaccttgaggcatacttcaaagactgtgtgtttactgagtgggaggagttgggggaggagattaggttaaaggtctttgtactaggaggctgtaggcataaattggtgtgttcaccagcaccatgcaactttttcacctctgcctaatcatctcatgttcatgtcctactgttcaagcctccaagctgtgccttgggtggctttggggcatggacattgacccgtataaagaatttggagcttctgcggagttactctcttttttaccttctgacttctttccttctattcgagatcttctcgacaccgcctctgctctgtatcgggaggccttagagtctccggaacattgttcacctcaccatacggcactcaggcaagctattctgtgttggggtgagttgatgaatctagccacctgggtgggaagtaatttggaagatccagcatccagggaattagtagtcggctatgtcaacgttaatatgggcctaaaacttagacaactattgtggtttcacatttcctgtcttacttttgggagagaaactgttcttgaatatttggtgtcttttggagtgtggattcgcactccttctgcatatagaccaccaaatgcccctatcctatcaacacttccggaaactactgttgttagacgaagaggcaggtcccctagaagaagaactccctcgcctcgcagacgaaggtctcaatcgccgcgtcgcagaagatctcaatctcgggaatctcaatgttagtattccttggacacataaggtgggaaactttacggggctttattcttctacggtaccttgttttaatcctaaatggcaaactccttcttttcctgacattcatttgcaggaggacattgttgatagatgtaagcaatttgtggggccccttacagtaaatgaaaacaggagactaaaattaattatgcctgctaggttttatcccaatgttactaaatatttgcccttagataaagggatcaaaccgtattatccagagtatgtagttaatcattacttccagacgcgacattatttacacactctttggaaagcggggatcttatataaaagagagtccactcgtagcgcctcattttgcgggtcaccatattcttgggaacaagatctacagcatgggaggttggtcttccaaacctcgaaaaggcatggggacaaatctttctgtccccaatcccctgggattcttccccgatcatcagttggaccctgcattcaaagccaactcagaaaatccagattgggacctcaacccgcacaaggacaactggccggacgccaacaaggtgggagtgggagcattcgggccagggttcacccctccccatggggggctgttggggtggagccctcaggctcagggcctactcacaactgtgccagcagctcctcctcctgcctccaccaatcggcagtcaggaaggcagcctactcccttatctccacctctaagggacactcatcctcaggccatgaagtgg

SEQ ID NO: 43 - DNA, 3215 bp, Hepatitis B virus
aattccacaacattccaccaagctctgctagaccccagagtgaggggcctatactttcctgctggtggctccagttccggaacagtaaaccctgttccgactactgcctcacccatatcgtcaatcttctcgaggactggggaccctgcaccgaacatggagagcacaacatcaggattcctaggacccctgctcgtgttacaggcggggtttttcttgttgacaagaatcctcacaataccacagagtctagactcgtggtggacttctctcaattttctagggggagcacccacgtgtcctggccaaaattcgcagtccccaacctccaatcactcaccaacctcttgtcctccaatttgtcctggctatcgctggatgtgtctgcggcgttttatcatattcctcttcatcctgctgctatgcctcatcttcttgttggttcttctggactaccaaggtatgttgcccgtttgtcctctacttccaggaacatcaactaccagcacgggaccatgcaagacctgcacgagtcctgctcaaggaacctctatgtttccctcttgttgctgtacaaaaccttcggacggaaactgcacttgtattcccatcccatcatcctgggctttcgcaagattcctatgggagtgggcctcagtccgtttctcctggctcagtttactagtgccatttgttcagtggttcgtagggctttcccccactgtttggctttcagttatatggatgatgtggtattgggggccatgtctgtacaacatcttgagtccctttttacctctattaccaattttcttttgtctttgggtatacatttgaaccctaataaaaccaaacgttggggctactcccttaacttcatgggatatgtaattggaagttggggtactttaccgcaagaacatattgtacaaaaacttaagcaatgttttcgaaaactgcctgtaaatagacctattgattggaaagtatgtcagagaattgtgggtcttttgggctttgctgccccttttacacaatgtggctatcctgctttaatgcctttatatgcatgtatacaatctaagcaggctttcactttctcgccaacttacaaggcctttctgtgtaaacaatatctgaacctttaccccgttgcccggcaacggtcaggtctctgccaagtgtttgctgacgcaacccccactggatggggcttggctattggccatcgccgcatgcgtggaacctttgtggctcctctgccgatccatactgcggaactcctagcagcttgttttgctcgcagccggtctggagcaaaacttatcggcaccgacaactctgttgtcctctctcggaagtacacctcctttccatggctgctagggtgtgctgccaactggatcctgcgcgggacgtcctttgtttacgtcccgtcggcgctgaatcccgcggacgacccgtctcggggccgtttgggactctaccgtccccttcttcatctgccgttccggccgaccacggggcgcacctctctttacgcggtctccccgtctgtgccttctcatctgccggaccgtgtgcacttcgcttcacctctgcacgtcgcatggagaccaccgtgaacgcccaccaggtcttgcccaaggtcttacataagaggactcttggactctcagcaatgtcaacgaccgaccttgaggcatacttcaaagactgtttgtttaaggactgggaggagttgggggaggagattaggttaaaggtctttgtactaggaggctgtaggcataaattggtctgttcaccagcaccatgcaactttttcacctctgcctaatcatctcatgttcatgtcctactgttcaagcctccaagctgtgccttgggtggctttggggcatggacattgacccgtataaagaatttggagcttctgtggagttactctcttttttgccttctgacttctttccttctattcgagatctcctcgacaccgcctctgctctgtatcgggaggccttagagtctccggaacattgttcgcctcaccatacagcactcaggcaagctattctttgttggggtgagttgatgaatctggccacctgggtgggaagtaatttggaagacccagcatccagggaattagtagccagctatgtcaatgttaatatgggcctaaaaatcagacaactactgtggtttcacatttcctgtcttacttttggaagagaaactgttcttgagtatttggtatcttttggagtgtggattcgcactcctcctgcttacagaccaccaaatgcccctatcttatcaacacttccggaaactactgttgttagacgacgaggcaggtcccctagaagacgaactccctcgcctcgcagacgaaggtctcaatcgccgcgtcgcagaagatctcaatctcgggaatctcaatgttagtatcccttggactcataaggtgggaaactttactgggctttattcttctactgtacctgtctttaatccagagtggcaaactccctcctttcctcacattcatttacaggaggacattattaatagatgtcaacaatatgtgggccctcttacagttaatgaaaaaagaagattaaaattaattatgcctgctaggttctatcctaaccttaccaaatatttgcccttggacaaaggcattaaaccatattatcctgaacatgcagttaatcattacttcaaaactaggcattatttacatactctgtggaaggctggcattctatataagagagaaactacacgcagcgcctcattttgtgggtcaccatattcttgggaacaagagctacagcatgggaggttggtcttccaaacctcgacaaggcatggggacaaatctttctgttcccaatcctctgggattctttcccgatcaccagttggaccctgcgttcggagccaactcaaacaatccagattgggacttcaaccccaacaaggatcactggccagaggcaaatcaggtaggagcgggagcattcgggccagggttcaccccaccacacggcggtcttttggggtggagccctcaggctcagggcatactgacaacagtgccagtagcacctcctcctgcctccaccaatcggcagtcaggaagacagcctactcccatctctccacctctaagagacagtcatcctcaggccatgcagtgg

SEQ ID NO: 44 - DNA, 3182 bp, Hepatitis B virus
aactccacaaccttccaccaaactctgcaagatcccagagtgagaggcctgtatttccctgctggtggctccagttcaggaacagtaaaccctgttccgactactgtctctcccatatcgtcaatcttctcgaggattggggaccctgcgctgaacatggagaacatcacatcaggattcctaggacccctgctcgtgttacaggcggggtttttcttgttgacaagaatcctcacaataccgcagagtctagactcgtggtggacttctctcaattttctagggggaactaccgtgtgtcttggccaaaattcgcagtccccaacctccaatcactcaccaacctcctgtcctccaacttgtcctggttatcgctggatgtgtctgcggcgttttatcatcttcctcttcatcctgctgctatgcctcatcttcttgttggttcttctggactatcaaggtatgttgcccgtttgtcctctaattccaggatcttcaactaccagcacgggaccatgcagaacctgcacgactcctgctcaaggaacctctatgtatccctcctgttgctgtaccaaaccttcggacggaaattgcacctgtattcccatcccatcatcctgggctttcggaaaattcctatgggagtgggcctcagcccgtttctcctggctcagtttactagtgccatttgttcagtggttcgtcgggctttcccccactgtttggctttcagttatatggatgatgtggtattgggggccaagtctgtacagcatcttgagtccctttttaccgctgttaccaattttcttttgtctttgggtatacatttaaaccctgacaaaacaaaaagatggggttactctttacatttcatgggctatgtcattggaagttatgggtcattgccacaagatcacatcatacaaaaaatcaaagaatgttttcgaaaacttcctgttaacagacctattgattggaaagtctgtcaacgtattgtgggtcttttgggttttgctgccccttttacacaatgtggttatcctgctttaaagcctttgtatgcatgtattcaatctaagcaggctttcactttctcgccaacttacaaggcctttctgtgtaaacaatacctgaacctttaccccgttgcccggcaacggccaggtctgtgccaagtgtttgctgacgcaacccccactggctggggcttggtcatgggccatcagcgcatgcgtggaacctttctggctcctctgccgatccatactgcggaactcctagccgcttgttttgctcgcagcaggtctggagcaaacattctcgggacggataactctgttgttctctcccgcaaatatacatcgtttccatggctgctaggctgtgctgccaactggatcctgcgcgggacgtcctttgtttacgtcccgtcggcgctgaatcccgcggacgacccttctcggggtcgcttgggactctctcgtccccttctccgtctgccgtttcgaccgaccacggggcgcacctctctttacgcggactccccgtctgtgccttctcatctgccggaccgtgtgcacttcgcttcacctctgcccgtcgcatggagaccaccgtgaacgcccaccgagtcttgcccaaggtcttacataagaggactcttggactctctgtaatgtcaacgaccgaccttgaggcatacttcaaagactgtttgttcaaagactgggaggagttgggggaggagattagattaaaggtctttgtactaggaggctgtaggcataaattggtctgcgcaccagcaccatgcaactttttcacctctgcctaatcatctcttgttcatgtcctactgttcaagcctccaagctgtgccttgggtggctttagggcatggacatcgatccttataaagaatttggagctactgtggagttactctcgtttttgccttctgacttctttccttcagtacgagatcttctagataccgcctcagctctgtatcgggaagccttagagtctcctgagcattgttcacctcaccatactgcactcaggcaagcagttctgtgctggggggaactaatgactctagctacctgggtgggtggtaatttggaagatccaacatccagggacctagtagtcagttatgtcaacactaatatgggcctaaagttccggcaactattgtggtttcacatttcttgtctcacttttggaagagaaacagttttagagtatttggtgtctttcggagtgtggattcgcactcctccagcttatagaccaccaaatgcccctatcttatcaacacttccggagactactgttgttagacgacgaggcaggtcccctagaagaagaactccctcgcctcgcagacgaaggtctcaatcgccgcgtcgcagaagatctcaatctcgggaatctcaatgttagtattccttggactcataaggtgggaaactttacggggctttattcttctactgtacctgtctttaaccctcattggaaaacaccctcttttcctaatatacatttacaccaagacattatcaaaaaatgtgaacaatttgtaggcccactcacagtcaatgaaaaaagaagactgcaattgattatgcctgctaggttttatccaaatgttaccaaatatttgccattggataagggtatcaaaccttattacccagaacatctagttaatcattacttccaaaccagacattatttacacactctatggaaggcgggtatattatataagagagaaacaacacatagcgcctcattttgtgggtcaccatattcttgggaacaaaagctacagcatggggcagaatctttccaccagcaatcctctgggattctttcccgaccaccagttggatccagccttcagagcaaacaccgcaaatccagattgggacttcaatcccaacaaggacacctggccagacgccaacaaggtaggagctggagcattcgggctgggattcaccccaccgcacggaggccttttggggtggagccctcaggctcagggcatactacaaaccttgccagcaaatccgcctcctgcctctacccatcgccagtcaggaaggcagcctaccccgctgtctccacctttgagaaacactcatcctcaggccatgcagtgg

SEQ ID NO: 45 - DNA, 3212 bp, Hepatitis B virus
ttccacagcattccaccaagctctgcaggatcccaaagtaagaggcctgtattttcctgctggtggctccagttccggaacagtgagccctgttccgactactgcctcactcatctcgtcaatcttctcgaggattggggaccctgcaccgaacatggaaggcatcacatcaggattcctgggacccctgctcgtgttacaggcggggtttttcttgttgacaaaaatcctcacaataccgcagagtctagactcgtggtggacttctctcaattttctagggggagctcccgtgtgtcttggccaaaattcgcagtccccaacctccaatcactcaccaacctcttgtcctccgatttgtcctggctatcgctggatgtgtctgcggcgttttatcatcttcctcttcatcctgctgctatgcctcatcttcttgttggttcttctggactatcaaggtatgttgcccgtttgtcctctaattccaggatcatcaaccaccagtacgggaccctgccgaacctgcacgactcttgctcaaggaacctctatgtttccctcatgttgctgttcaaaaccttcggacggaaattgcacttgtattcccatcccatcatcatgggctttcggaaaattcctatgggagtgggcctcagcccgtttctcctggctcagtttactagtgccatttgttcagtggttcgccgggctttcccccactgtctggctttcagttatatggatgatgtggtattgggggccaagtctgtacaacatcttgagtccctttatacctctgttaccaattttcttttgtctttgggtatacatttaaatcccaacaaaacaaaacgatggggatattctcttaatttcatgggatatgtaattgggagttgggggtcattaccacaggaacacatccgaatgaaaatcaaagactgttttagaaaactccctgttaaccggcctattgattggaaagtatgtcaaagaattgtgggtcttttgggctttgctgccccttttacacaatgtggatatcctgctttaatgcctctgtatgcgtgtgttcaatcgaagcaggctttcactttctcgccaacttacaaggcctttctgtgtaaacaatacctgaacctttaccccgttgcccggcaacggccaggtctgtgccaagtgtttgctgatgcaacccccactggctggggcttggccataggccatcagcgcatgcgtggaacctttgtggctcctctgccgatccatactgcggaactcctagccgcttgttttgctcgcagcaggtctggagcgaaacttatcgggacggataattctgtcgttctctcccggaaatatacatcatttccatggctgctaggctgtgctgccaactggatcctgcgagggacgtcctttgtctacgtcccgtcagcgctgaatcctgcggacgacccgtctcggggtcgcttggggatctatcgtccccttctccgtctgccgttccggccgaccacggggcgcacctctctttacgcggtctccccgtctgtgccttctcatctgccggaccgtgtgcacttcgcttcacctctgcacgtcgcatggagaccaccgtgaacgcccatcaaatcttgcccaaggtcttacataagcggactcttggactttctgcaatgtcaacgaccgaccttgaggcatacttcaaagactgtttgtttaaagactgggaggagttgggggaggagattagattaaaggtctttgtactaggaggctgtaggcataaattggtctgcgcaccagcaccatgcaactttttcacctctgcctaatcatctcttgttcatgtcctactgttcaagcctccaagctgtgccttgggtggctttggggcatggacattgacccttataaagaatttggagctactgtggagttactctcgtttttgccgtctgacttctttccgtcagttagagatcttctagataccgcctcagctctgtatcgggatgccttagaatctcctgagcattgttcacctcaccatactgcactcaggcaagccattctttgctggggggaactaatgactctagctacctgggtgggtgtaaatttggaagatccagcatccagggacctagtagtcagttatgtcaatactaatatgggcctaaagttcaggcaattattgtggtttcacatttcttgtctcacttttggaagagaaaccgtcatagagtatttggtgtcttttggagtgtggattcgcactcctccagcttatagaccaccaaatgcccctatcttatcaacacttccggagaatactgttgttagacgaagaggcaggtcccctagaagaagaactccctcgcctcgcagacgaagatctcaatcgccgcgtcgcagaagatctcaatctccagcttcccaatgttagtattccttggactcacaaggtgggaaattttacgggcctttactcttctactatacctgtctttaatcctaactggaaaactccatcttttcctgatattcatttgcaccaagacattattaacaaatgtgaacaatttgtaggtcctctaacagtaaatgaaaaacgaagattaaacttagtcatgcctgctagattttttcccatctctacgaaatatttgcccctagagaagggtataaaaccttattatccagataatgtagttaatcattacttccaaaccagacactatttacataccctatggaaggcgggcatcttatataaacgggaaactacacgtagcgcctcattttgtgggtcaccttattcttgggaacaagagctacatcatggggctttcttggacggtccctctcgaatgggggaagaatcattccaccaccaatcctctgggattttttcccgaccaccagttggatccagcattcagagcaaacaccagaaatccagattgggaccacaatcccgacaaagaccactggacagaagccaacaaggtaggagtgggagcattcgggccggggttcactcccccacacggaggccttttggggtggagccctcaggctcaaggcatgctaaaaacattgccagcagatccgcctcctgcctccaccaatcggcagtcaggaaggcagcctaccccaatcactccacctttgagagacactcatcctcaggccatgcagtggaa

SEQ ID NO: 46 - DNA, 3215 bp, Hepatitis B virus
ctccactcagttccaccaggctctgttagatccgagagtaagggctctgtattttcctgctggtggctccagttcagagacacagaaccctgctccgactattgcctctctcacatcatcaatcttcttgaagactgggggccctgctacgaacatggacaacatcacatcaggactcctaggacccctgctcgtgttacaggcggtgtgtttcttgttgacaaaaatcctcacaataccacagagtctagactcgtggtggacttctctcaattttctagggggaacacccgggtgtcctggccaaaattcgcagtccccaacctccaatcacttaccaacctcctgtcctccaacttgtcctggctatcgctggatgtgtctgcggcgttttatcatcttcctcttcatcctgctgctatgcctcatcttcttgttggttcttctggactatcaaggtatgttgcccgtttgtcctctacttccaggatccacgaccaccagcacgggaccatgcaaaacctgcacaactcttgctcaaggaacctctatgtttccctcttgctgctgttccaaaccctcggacggaaactgcacttgtattcccatcccatcatcctgggctttaggaaaatacctatgggagtgggcctcagcccgtttctcctggctcagtttactagtgcaatttgttcagtggtgcgtagggctttcccccactgtctggcttttagttatatggatgatctggtattgggggccaaatctgtgcagcatcttgagtccctttataccgctgttaccaattttctgttatctgtgggtatccatttaaatacctcgaaaacaaaaagatggggttataccctaaatttcatgggttatgttattggcagttggggatcattaccacaagatcacattgtacaaaaaatcaaagattgttttcgtaaacttcctgtaaatcgccctattgattggaaagtttgtcaacgcattgtgggtcttttgggctttgccgccccctttactcaatgtggttatcctgctctcatgcctctgtatgcctgtataactgctaaacaggcttttgtcttttcgccaacttacaaggcctttctatgtcaacaatacatgaacctttaccccgttgctcggcaacggccaggcctgtgccaagtgtttgctgacgcaacccccactggttggggcttggccattggccatcagcgcatgcgtggaacctttgtggctcctctgccgatccatactgcggaactccttgcagcttgtttcgctcgcagccggtctggagcgaaactcatcggcacagacaactctgttgtcctctctaggaagtacacctccttcccatggctgctcggttgtgctgccaactggatcctacgcgggacgtcctttgtttacgtcccgtcggcgctgaatccagcggacgatccctctcggggtcgcttggggctgtatcgcccccttctccgtctgccgttccagccgacgacgggtcgcacctctctttacgcggcctccccgtctgttccttctcgtctgccggaccgtgtgcacttcgcttcacctctgcacgtcgcatggagaccaccgtgaacgcccctcgaagcttgccaacagtcttacataagcggactcttggactttcaggaaggtcaatcacctggatcgaagaatacatcaaagactgtgtatttaaggactgggaggagctgggggaggagattaggttaaaggtctttgtattaggaggctgtaggcataaattggtctgttcaccagcaccatgcaactttttcacctctgcctaatcatcttttgttcatgtcctactgttcaagcctccaagctgtgccttgggtggctttggggcatggacattgacccttataaagaatttggagcttctgtggaattactctcttttttgccttctgacttcttcccgtcagttcgggacctactcgacaccgcttcagccctctaccgggatgctttagaatcaccagaacattgcacacctaaccataccgctctcaggcaagctatattgtgctggggtgagttaatgactttggcttcctgggtgggcaataacttggaagatcctgctgctagggacctagtggttaactatgtcaatactaacatgggcctaaaaattagacaattgctgtggtttcacatttcctgccttacttttggaagagaaacagttcttgagtatttggtgtcttttggagtgtggattcgcactcctcctgcttatagaccaccaaatgcccctatcttatccacacttccggaaactactgttgttagacgacgaggcaggtcccctcgaagaagaactccctcgcctcgcagacgaaggtctcaatcgccgcgtcgcagaagatctcaatctccagcttcccaatgttagtattccttggactcataaggtgggaaattttacgggactctattcctctactgttcctacttttaatcctgactggttaactccttcttttcctgacattcatttacatcaagatttgatacacaaatgtgaacaatttgtaggccctctcacaaaaaatgaattgagaagattaaaattagttatgccatccagattttttcctaaggttaccaaatattttcctatggaaaagggaattaaaccctattatcctgataacgtggttaatcattattttaagaccagacactatttgcatactttatggaargcrggcattctatataagagagaatccacacgtagcgcctcattttgtgggtcaccatattcttgggaacaagagctacagcatgggagcacctctatcaacgactcgaaggggcatgggacagaatctctctgtacccaatcctctgggattctttccagaccatcagctggatcctctattcagggcaaattccagcagtcccgactgggacttcaacaaaaacaaggacaattggccaatggcaaacaaggtaggagtgggaggatacggtcctgggttcacacccccacacggtggcctgttggggtggagtccacaggcacagggtgtgcttacaacattgccagcagatccgcctcctgcttccaccaatcggcggtccgggagaaaaccaaccccagtctctccacctctaagagacactcatccacaggccatgcagtggaa

SEQ ID NO: 47 - DNA, 3248 bp, Hepatitis B virus
ctctacagcattccaccaagctctacaaaatcccaaagtcaggggcctgtattttcctgctggtggctccagttcagggatagtgaaccctgttccgactattgcctctcacatctcgtcaatcttctccaggattggggaccctgcaccgaacatggagaacatcacatcaggattcctaggacccctgctcgtgttacaggcggggtttttcttgttgacaagaatcctcacaataccgcagagtctagactcgtggtggacttctctcaattttctagggggagtgcccgtgtgtcctggcctaaattcgcagtccccaacctccaatcactcaccaatctcctgtcctccaacttgtcctggctatcgctggatgtgtctgcggcgttttatcatattcctcttcatcctgctgctatgcctcatcttcttgttggttcttctggactatcaaggtatgttgcccgtttgtcctctgattccaggatcctcgaccaccagcacgggaccctgcaaaacctgcacgactcctgctcaaggcaactctatgtatccctcatgttgctgtacaaaaccttcggacggaaattgcacctgtattcccatcccatcatcttgggctttcgcaaaatacctatgggagtgggcctcagtccgtttctcttggctcagtttactagtgccatttgttcagtggttcgtagggctttcccccactgtctggctttcagctatatggatgatgtggtattgggggccaaatctgtacaacatcttgagtccctttataccgctgttaccaattttcttttgtctttgggtatacatctaaaccctaacaaaacaaaaagatggggttattccttaaattttatgggatatgtaattggaagttggggtactttgccacaagaacacatcacacagaaaattaagcaatgttttcggaaactccctgttaacaggccaattgattggaaagtctgtcaacgaataactggtctgttgggtttcgctgctccttttacccaatgtggttaccctgccttaatgcctttatatgcatgtatacaagctaagcaggcttttactttctcgccaacttataaggcctttctctgtaaacaatacatgaacctttaccccgttgctaggcaacggcccggtctgtgccaagtgtttgctgacgcaacccccactggttggggcttggccatcggccatcagcgcatgcgtggaacctttgtggctcctctgccgatccatactgcggaactcctagctgcttgttttgctcgcagccggtctggagcaaaactcattgggactgacaattctgtcgtcctttctcggaaatatacatcctttccatggctgctaggctgtgctgccaactggatccttcgcgggacgtcctttgtttacgtcccgtcagcgctgaatccagcggacgacccctcccggggccgtttggggctctgtcgcccccttctccgtctgccgttcctgccgaccacggggcgcacctctctttacgcggtctccccgtctgttccttctcatctgccggaccgtgtgcacttcgcttcacctctgcacgttacatggaaaccgccatgaacacctctcatcatctaccaaggcagttatataagaggactcttggactgtttgttatgtcaacaaccgggatggagaaatacttcaaggactgtgtttttgctgagtgggaagaattaggcaatgagtccaggttaatgacctttgtattaggaggctgtaggcataaattggtctgcgcaccagcaccatgtaactttttcacctctgcctaatcatctcttgttcatgtcctactgttcaagcctccaagctgtgccttgggtggctttagggcatggatagaacaactttgccatatggcctttttggcttagacattgacccttataaagaatttggagctactgtggagttgctctcgtttttgccttctgactttttcccgtctgttcgtgatcttctcgacaccgcttcagctttgtaccgggaatccttagagtcctctgatcattgttcgcctcaccatacagcactcaggcaagcaattctgtgctggggtgagttgatgactctagctacctgggtgggtaataatttggaagatccagcatccagagatttggtggtcaattatgttaatactaatatgggtttaaaaatcaggcaactattgtggtttcacatttcctgtcttacttttgggagagaaaccgttcttgagtatttggtgtcttttggagtgtggattcgcactcctcctgcttatagaccaccaaatgcccctatcctatcaacacttccggagactactgttgttagacgaagaggcaggtcccctcgaagaagaactccctcgcctcgcagacgaagatctcaatcgccgcgtcgcagaagatctgcatctccagcttcccaatgttagtattccttggactcacaaggtgggaaactttacggggctgtattcttctactatacctgtctttaatcctgattggcaaactccttcttttccaaatatccatttgcatcaagacattataactaaatgtgaacaatttgtgggccctctcacagtaaatgagaaacgaagattaaaactagttatgcctgccagatttttcccaaactctactaaatatttaccattagacaaaggtatcaaaccgtattatccagaaaatgtagttaatcattacttccagaccagacattatttacataccctttggaaggcgggtattctatataagagagaaacatcccgtagcgcttcattttgtgggtcaccatatacttgggaacaagatctacagcatggggctttcttggacggtccctctcgagtggggaaagaacctttccaccagcaatcctctaggattccttcccgatcaccagttggacccagcattcagagcaaataccaacaatccagattgggacttcaatcccaaaaaggacccttggccagaggccaacaaggtaggagttggagcctatggacccgggttcacccctccacacggaggccttttggggtggagccttcagtctcagggcacactaacaactttgccagcagatccgcctcctgcctccaccaatcgtcagtcagggaggcagcctactcccatctctccaccactaagagacagtcatcctcaggccatgcagtggaa

SEQ ID NO: 48 - DNA, 3215 bp, Hepatitis B virus
ctcaacacagttccaccaagcactgttggatccgagagtaagggggctgtattttcctgctggtggctccagttcagaaacacagaaccctgctccgactattgcctctctcacatcatcaatcttctcgaagactggggaccctgctatgaacatggagaacatcacatcaggactcctaggaccccttctcgtgttacaggcggtgtgtttcttgttgacaaaaatcctcacaataccaaagagtctagactcgtggtggacttctctcaattttctaggggtaccacccgggtgtcctggccaaaattcgcagtccccaatctccaatcacttaccaacctcctgtcctccaacttgtcctggctatcgttggatgtgtctgcggcgttttatcatcttcctcttcatcctgctgctatgcctcatcttcttgttggttcttctggactatcaaggtatgttgcccgtgtgtcctctacttccaggatcwacaaccaccagcacgggaccctgcaaaacctgcaccactcttgctcaaggaacctctatgtttccctcctgctgctgtaccaaaccttcggacggaaattgcacctgtattcccatcccatcatcttgggctttcggaaaatacctatgggagtgggcctcagcccgtttctcttggctcagtttactagtgcaatttgttcagtggtgcgtagggctttcccccactgtctggcttttagttatatggatgatctggtattgggggccaaatctgtgcagcatcttgagtccctttataccgctgttaccaattttttgttatctgtgggcatccatttgaacacagctaaaacaaaatggtggggttattcccttcactttatgggttatataattgggagttgggggaccttgcctcaggaacatattgtgcataaaatcaaagattgctttcgcaaacttcccgtgaatagacccattgattggaaggtttgtcaacgcattgtgggtcttttgggctttgcagccccttttactcaatgtggttatcctgctctcatgcccttgtatgcctgtattrccgctaagcaggcttttgttttctcgccaacttacaaggcctttctctgtaaacaatacatgaacctttaccccgttgctcggcaacggccaggcctttgccaagtgtttgctgacgcaacccccactggctggggcttggcgattggccatcagcgcatgcgcggaacctttgtggctcctctgcccatccatactgcggaactcctagccgcttgtttcgctcgcagcaggtctggagcggacattatcggcactgacaactccgttgtcctttctcggaagtacacctccttcccatggctgctaggctgtgctgccaactggatcctgcgcgggacgtcctttgtctacgtcccgtcggcgctgaatcctgcggacgacccctctcgtggtcgcttggggctctgccgccctcttctccgcctgccgttccggccgacgacgggtcgcacctctctttacgcggactccccgcctgtgccttctcatctgccggcccgtgtgcacttcgcttcacctctgcacgtcgcatggagaccaccgtgaacgccccttggaacttgccaacaaccttacataagaggactcttggactttcgccccggtcaacgacctggattgaggaatacatcaaagactgtgtatttaaggactgggaggagtcgggggaggagttgaggttaaaggtctttgtattaggaggctgtaggcataaattggtctgttcaccagcaccatgcaactttttcacctctgcctaatcatcttttgttcatgtcccactgttcaagcctccaagctgtgccttgggtggctttggggcatggacattgacccttataaagaatttggagcttctgtggagttactctcatttttgccttctgacttcttcccgtctgtccgggacctactcgacaccgcttcagccctctaccgagatgccttagaatcaccagaacattgcacccccaaccacactgctctcaggcaagctattttgtgctggggtgagttgatgaccttggcttcctgggtgggcaataatttagaggatcctgcagcaagagatctagtagttaattatgtcaatactaacatgggcctaaaaattagacaattattatggtttcacatttcttgccttacatttggaagagaaactgtgcttgagtatttggtgtcttttggagtgtggattcgcactccacctgcttatagaccaccaaatgcccctatcctatcaacacttccggagactactgttgttagacaacgaggcagggcccctagaagaagaactccctcgcctcgcagacgaagatctcaatctccgcgtcgcagaagatctcaatctccagcttcccaatgttagtattccttggactcataaggtgggaaactttaccggtctttactcctctactatacctgttttcaatcctgactggttaactccttcttttcctgacattcacttgcatcaagatctgatacaaaaatgtgaacaatttgtaggcccactcactacaaatgaaaggagacgattgaaactaattatgccagctaggttttatcccaaagttactaaatacttccctttggataaaggtattaagccttactatccagagaatgtggttaatcattactttaaaactagacattatttacatactttgtggaaggcaggaattctatataagagagaatccacacatagcgcctcattttgtgggtcaccatattcctgggaacaagagctacagcatgggagcacctctctcaacggcgagaaggggcatgggacagaatctttctgtgcccaatcctctgggattctttccagaccaccagttggatccactattcagagcaaattccagcagtcccgattgggacttcaacacaaacaaggacaattggccaatggcaaacaaggtaggagtgggaggcttcggtccagggttcacacccccacacggtggccttctggggtggagccctcaggcacagggcattctaacaacctcgccaccagatccacctcctgcttccaccaatcggaggtcaggaagaaagccaaccccagtctctccacctctaagggacacacatccacaggccatgcagtggaa

SEQ ID NO: 50 - protein, 47 aa, Artificial Sequence
GTNLSVPNPLGFFPDHQLDPAFGANSNNPDWDFNPNKDHWPEANKVG

SEQ ID NO: 50 - protein, 47 aa, Artificial Sequence
  PEPTIDE (1)..(47): Synthetic polypeptide
  MYRISTATE (1)..(1): N-term Myr
  AMIDATION (47)..(47): C-term NH2
GLNQSTFNPLGFFPSHQLDPLFKANAGSADWDKNPNKDPWPQAHDTA

SEQ ID NO: 51 - protein, 47 aa, Artificial Sequence; identical to SEQ ID NO: 50
  PEPTIDE (1)..(47): Synthetic polypeptide
  MYRISTATE (1)..(1): N-term Myr
  AMIDATION (47)..(47): C-term NH2